European Patent Application EP 4 501 965 A1, published February 5, 2025. Title: 抗体、融合蛋白及其用途. Applicant: 成都地奥制药集团有限公司. The sequence listing filed with the application follows.

SEQUENCE LISTING (97 sequences)

SEQ ID NO: 1 - protein, 11 aa, synthetic construct
RASQGVGTAVA

SEQ ID NO: 2 - protein, 7 aa, synthetic construct
SASGLYS

SEQ ID NO: 3 - protein, 9 aa, synthetic construct
QQHGTTPPT

SEQ ID NO: 4 - protein, 10 aa, synthetic construct
GFNIGGTGIH

SEQ ID NO: 5 - protein, 15 aa, synthetic construct
GIYPTNGGTGYAGSV

SEQ ID NO: 6 - protein, 11 aa, synthetic construct
GGGDGFGAMGY

SEQ ID NO: 7 - protein, 11 aa, synthetic construct
GGGGSGGGGSA

SEQ ID NO: 8 - protein, 7 aa, synthetic construct
GGGGSGS

SEQ ID NO: 9 - protein, 9 aa, synthetic construct
GGGGSGGGG

SEQ ID NO: 10 - protein, 10 aa, synthetic construct
GGGGSGGGGS

SEQ ID NO: 11 - protein, 15 aa, synthetic construct
GGGGSGGGGSGGGGS

SEQ ID NO: 12 - protein, 11 aa, synthetic construct
GGGGSGGGGSY

SEQ ID NO: 13 - protein, 107 aa, synthetic construct
DIQMTQSPSSLSASVGDRVTITCRASQGVGTAVAWYQQKPGKAPKLLIYSASGLYSGVPSRFSGSRSGTDFTLTISSLQPEDFATYYCQQHGTTPPTFGQGTKVEIK

SEQ ID NO: 14 - protein, 107 aa, synthetic construct
DIQMTQSPSSLSASVGDRVTITCGGGGSGGGGSAWYQQKPGKAPKLLIYGGGGSGSGVPSRFSGSRSGTDFTLTISSLQPEDFATYYCGGGGSGGGGFGQGTKVEIK

SEQ ID NO: 15 - protein, 118 aa, synthetic construct
EVQLVESGGGLVQPGGSLRLSCAASGFNIGGTGIHWVRQAPGKGLEWVAGIYPTNGGTGYAGSVKGRFTISADTSKNTAYLQMNSLRAEDTAVYYCSRGGGDGFGAMGYWGQGTLVTV

SEQ ID NO: 16 - protein, 118 aa, synthetic construct
EVQLVESGGGLVQPGGSLRLSCAASGGGGSGGGGSWVRQAPGKGLEWVAGGGGSGGGGSGGGGSKGRFTISADTSKNTAYLQMNSLRAEDTAVYYCSRGGGGSGGGGSYWGQGTLVTV

SEQ ID NO: 17 - protein, 450 aa, synthetic construct
EVQLVESGGGLVQPGGSLRLSCAASGFNIGGTGIHWVRQAPGKGLEWVAGIYPTNGGTGYAGSVKGRFTISADTSKNTAYLQMNSLRAEDTAVYYCSRGGGDGFGAMGYWGQGTLVTVSSASTKGPSVFPLAPSSKSTSGGTAALGCLVKDYFPEPVTVSWNSGALTSGVHTFPAVLQSSGLYSLSSVVTVPSSSLGTQTYICNVNHKPSNTKVDKKVEPKSCDKTHTCPPCPAPELLGGPSVFLFPPKPKDTLMISRTPEVTCVVVDVSHEDPEVKFNWYVDGVEVHNAKTKPREEQYNSTYRVVSVLTVLHQDWLNGKEYKCKVSNKALPAPIEKTISKAKGQPREPQVYTLPPSRDELTKNQVSLTCLVKGFYPSDIAVEWESNGQPENNYKTTPPVLDSDGSFFLYSKLTVDKSRWQQGNVFSCSVMHEALHNHYTQKSLSLSPGK

SEQ ID NO: 18 - protein, 450 aa, synthetic construct
EVQLVESGGGLVQPGGSLRLSCAASGGGGSGGGGSWVRQAPGKGLEWVAGGGGSGGGGSGGGGSKGRFTISADTSKNTAYLQMNSLRAEDTAVYYCSRGGGGSGGGGSYWGQGTLVTVSSASTKGPSVFPLAPSSKSTSGGTAALGCLVKDYFPEPVTVSWNSGALTSGVHTFPAVLQSSGLYSLSSVVTVPSSSLGTQTYICNVNHKPSNTKVDKKVEPKSCDKTHTCPPCPAPELLGGPSVFLFPPKPKDTLMISRTPEVTCVVVDVSHEDPEVKFNWYVDGVEVHNAKTKPREEQYNSTYRVVSVLTVLHQDWLNGKEYKCKVSNKALPAPIEKTISKAKGQPREPQVYTLPPSRDELTKNQVSLTCLVKGFYPSDIAVEWESNGQPENNYKTTPPVLDSDGSFFLYSKLTVDKSRWQQGNVFSCSVMHEALHNHYTQKSLSLSPGK

SEQ ID NO: 19 - protein, 214 aa, synthetic construct
DIQMTQSPSSLSASVGDRVTITCRASQGVGTAVAWYQQKPGKAPKLLIYSASGLYSGVPSRFSGSRSGTDFTLTISSLQPEDFATYYCQQHGTTPPTFGQGTKVEIKRTVAAPSVFIFPPSDEQLKSGTASVVCLLNNFYPREAKVQWKVDNALQSGNSQESVTEQDSKDSTYSLSSTLTLSKADYEKHKVYACEVTHQGLSSPVTKSFNRGEC

SEQ ID NO: 20 - protein, 214 aa, synthetic construct
DIQMTQSPSSLSASVGDRVTITCGGGGSGGGGSAWYQQKPGKAPKLLIYGGGGSGSGVPSRFSGSRSGTDFTLTISSLQPEDFATYYCGGGGSGGGGFGQGTKVEIKRTVAAPSVFIFPPSDEQLKSGTASVVCLLNNFYPREAKVQWKVDNALQSGNSQESVTEQDSKDSTYSLSSTLTLSKADYEKHKVYACEVTHQGLSSPVTKSFNRGEC

SEQ ID NO: 21 - protein, 347 aa, synthetic construct
EGVAAALTPERLLEWQDKGIFVIQSESLKKCIQAGKSVLTLENCKQANKHMLWKWVSNHGLFNIGGSGCLGLNFSAPEQPLSLYECDSTLVSLRWRCNRKMITGPLQYSVQVAHDNTVVASRKYIHKWISYGSGGGDICEYLHKDLHTIKGNTHGMPCMFPFQYNHQWHHECTREGREDDLLWCATTSRYERDEKWGFCPDPTSAEVGCDTIWEKDLNSHICYQFNLLSSLSWSEAHSSCQMQGGTLLSITDETEENFIREHMSSKTVEVWMGLNQLDEHAGWQWSDGTPLNYLNWSPEVNFEPFVEDHCGTFSSFMPSAWRSRDCESTLPYICKKYLNHIDHEIVE

SEQ ID NO: 22 - protein, 490 aa, synthetic construct
EGVAAALTPERLLEWQDKGIFVIQSESLKKCIQAGKSVLTLENCKQANKHMLWKWVSNHGLFNIGGSGCLGLNFSAPEQPLSLYECDSTLVSLRWRCNRKMITGPLQYSVQVAHDNTVVASRKYIHKWISYGSGGGDICEYLHKDLHTIKGNTHGMPCMFPFQYNHQWHHECTREGREDDLLWCATTSRYERDEKWGFCPDPTSAEVGCDTIWEKDLNSHICYQFNLLSSLSWSEAHSSCQMQGGTLLSITDETEENFIREHMSSKTVEVWMGLNQLDEHAGWQWSDGTPLNYLNWSPEVNFEPFVEDHCGTFSSFMPSAWRSRDCESTLPYICKKYLNHIDHEIVEKDAWKYYATHCEPGWNPYNRNCYKLQKEEKTWHEALRSCQADNSALIDITSLAEVEFLVTLLGDENASETWIGLSSNKIPVSFEWSNDSSVIFTNWHTLEPHIFPNRSQLCVSAEQSEGHWKVKNCEERLFYICKKAGHVLSD

SEQ ID NO: 23 - protein, 10 aa, synthetic construct
GGGGSGGGGS

SEQ ID NO: 24 - protein, 225 aa, synthetic construct
THTCPPCPAPELLGGPSVFLFPPKPKDTLMISRTPEVTCVVVDVSHEDPEVKFNWYVDGVEVHNAKTKPREEQYNSTYRVVSVLTVLHQDWLNGKEYKCKVSNKALPAPIEKTISKAKGQPREPQVYTLPPSRDELTKNQVSLTCLVKGFYPSDIAVEWESNGQPENNYKTTPPVLDSDGSFFLYSKLTVDKSRWQQGNVFSCSVMHEALHNHYTQKSLSLSPGK

SEQ ID NO: 25 - DNA, 1350 bp, synthetic construct
  source 1..1350: mol_type = other DNA
gaagtccagctggtggaaagtggcggtggactggttcaaccaggaggaagcctaagactaagctgcgccgccagcggttttaacatcggtggcacaggcatccattgggtccggcaggcacccggcaaaggtttagagtgggtcgcaggcatctaccccactaatggtggcaccggctacgctggtagcgtgaagggcaggttcaccattagcgctgacaccagcaagaacactgcttatctgcagatgaatagcctgcgtgccgaagacacagccgtctattactgtagtagaggcggaggtgatgggttcggcgcgatgggctactggggacagggcacactcgtgaccgttagtagcgctagcaccaagggcccatcggtcttccccctggcaccctcctccaagagcacctctgggggcacagcggccctgggctgcctggtcaaggactacttccccgaaccggtgacggtgtcgtggaactcaggcgccctgaccagcggcgtgcacaccttcccggctgtcctacagtcctcaggactctactccctcagcagcgtggtgaccgtgccctccagcagcttgggcacccagacctacatctgcaacgtgaatcacaagcccagcaacaccaaggtggacaagaaagtagagcccaaatcttgtgacaaaactcacacatgcccaccgtgcccagcacctgaactcctggggggaccgtcagtcttcctcttccccccaaaacccaaggacaccctcatgatctcccggacccctgaggtcacatgcgtggtggtggacgtgagccacgaagaccctgaggtcaagttcaactggtacgtggacggcgtggaggtgcataatgccaagacaaagccgcgggaggagcagtacaacagcacgtaccgtgtggtcagcgtcctcaccgtcctgcaccaggactggctgaatggcaaggagtacaagtgcaaggtctccaacaaagccctcccagcccccatcgagaaaaccatctccaaagccaaagggcagccccgagaaccacaggtgtacaccctgcccccatcccgggatgagctgaccaagaaccaggtcagcctgacctgcctggtcaaaggcttctatcccagcgacatcgccgtggagtgggagagcaatgggcagccggagaacaactacaagaccacgcctcccgtgctggactccgacggctccttcttcctctacagcaagctcaccgtggacaagagcaggtggcagcaggggaacgtcttctcatgctccgtgatgcatgaggctctgcacaaccactacacgcagaagagcctctccctgtctccgggtaaa

SEQ ID NO: 26 - DNA, 642 bp, synthetic construct
  source 1..642: mol_type = other DNA
gatatacagatgacgcagagccctagcagtctaagtgcaagcgttggagaccgtgtcaccattacctgccgcgctagccagggcgtcggcaccgcagtcgcctggtatcagcaaaaaccgggtaaggctccaaagctgttgatctacagtgccagcggcctgtacagcggtgtgccaagtaggttcagcgggagccggagtgggacagactttacactcactattagcagtctgcagcccgaggacttcgccacctactactgtcagcagcatggcacaacacccccaacattcgggcagggaaccaaagttgagataaaacgaacggttgccgcgccaagcgtatttatctttccccccagtgatgagcaactgaagagtggtacagccagcgttgtctgccttttgaataacttctatcctcgggaggcaaaggtccagtggaaagtggataatgcactccaaagcggtaacagccaggagagtgtgacagaacaggacagcaaagatagtacctacagcctcagtagtaccctcacactgagcaaagcggactatgaaaagcacaaggtgtacgcttgtgaagtgacccaccagggcctaagcagccctgttactaagagcttcaacagaggcgaatgt

SEQ ID NO: 27 - DNA, 1350 bp, synthetic construct
  source 1..1350: mol_type = other DNA
gaagtccagctggtggaaagtggcggtggactggttcaaccaggaggaagcctaagactaagctgcgccgccagcggtggcgggggtagcggtggcgggggttcgtgggtccggcaggcacccggcaaaggtttagagtgggtcgcaggtggcgggggtagcggtggcgggggttcgggcgggggtggttccaagggcaggttcaccattagcgctgacaccagcaagaacactgcttatctgcagatgaatagcctgcgtgccgaagacacagccgtctattactgtagtagaggcggaggtggtagcggtggcgggggttcgtactggggacagggcacactcgtgaccgttagtagcgctagcaccaagggcccatcggtcttccccctggcaccctcctccaagagcacctctgggggcacagcggccctgggctgcctggtcaaggactacttccccgaaccggtgacggtgtcgtggaactcaggcgccctgaccagcggcgtgcacaccttcccggctgtcctacagtcctcaggactctactccctcagcagcgtggtgaccgtgccctccagcagcttgggcacccagacctacatctgcaacgtgaatcacaagcccagcaacaccaaggtggacaagaaagtagagcccaaatcttgtgacaaaactcacacatgcccaccgtgcccagcacctgaactcctggggggaccgtcagtcttcctcttccccccaaaacccaaggacaccctcatgatctcccggacccctgaggtcacatgcgtggtggtggacgtgagccacgaagaccctgaggtcaagttcaactggtacgtggacggcgtggaggtgcataatgccaagacaaagccgcgggaggagcagtacaacagcacgtaccgtgtggtcagcgtcctcaccgtcctgcaccaggactggctgaatggcaaggagtacaagtgcaaggtctccaacaaagccctcccagcccccatcgagaaaaccatctccaaagccaaagggcagccccgagaaccacaggtgtacaccctgcccccatcccgggatgagctgaccaagaaccaggtcagcctgacctgcctggtcaaaggcttctatcccagcgacatcgccgtggagtgggagagcaatgggcagccggagaacaactacaagaccacgcctcccgtgctggactccgacggctccttcttcctctacagcaagctcaccgtggacaagagcaggtggcagcaggggaacgtcttctcatgctccgtgatgcatgaggctctgcacaaccactacacgcagaagagcctctccctgtctccgggtaaa

SEQ ID NO: 28 - DNA, 642 bp, synthetic construct
  source 1..642: mol_type = other DNA
gatatacagatgacgcagagccctagcagtctaagtgcaagcgttggagaccgtgtcaccattacctgcggtggcgggggtagcggtggcgggggttcggcctggtatcagcaaaaaccgggtaaggctccaaagctgttgatctacggtggcgggggtagcggcagcggtgtgccaagtaggttcagcgggagccggagtgggacagactttacactcactattagcagtctgcagcccgaggacttcgccacctactactgtggtggcgggggtagcggtggcgggggtttcgggcagggaaccaaagttgagataaaacgaacggttgccgcgccaagcgtatttatctttccccccagtgatgagcaactgaagagtggtacagccagcgttgtctgccttttgaataacttctatcctcgggaggcaaaggtccagtggaaagtggataatgcactccaaagcggtaacagccaggagagtgtgacagaacaggacagcaaagatagtacctacagcctcagtagtaccctcacactgagcaaagcggactatgaaaagcacaaggtgtacgcttgtgaagtgacccaccagggcctaagcagccctgttactaagagcttcaacagaggcgaatgt

SEQ ID NO: 29 - protein, 450 aa, synthetic construct
QVQLQQPGAELVKPGASVKMSCKASGYTFTSYNMHWVKQTPGRGLEWIGAIYPGNGDTSYNQKFKGKATLTADKSSSTAYMQLSSLTSEDSAVYYCARSTYYGGDWYFNVWGAGTTVTVSAASTKGPSVFPLAPSSKSTSGGTAALGCLVKDYFPEPVTVSWNSGALTSGVHTFPAVLQSSGLYSLSSVVTVPSSSLGTQTYICNVNHKPSNTKVDKKAEPKSCDKTHTCPPCPAPELLGGPSVFLFPPKPKDTLMISRTPEVTCVVVDVSHEDPEVKFNWYVDGVEVHNAKTKPREEQYNSTYRVVSVLTVLHQDWLNGKEYKCKVSNKALPAPIEKTISKAKGQPREPQVYTLPPSRDELTKNQVSLTCLVKGFYPSDIAVEWESNGQPENNYKTTPPVLDSDGSFFLYSKLTVDKSRWQQGNVFSCSVMHEALHNHYTQKSLSLSPG

SEQ ID NO: 30 - protein, 213 aa, synthetic construct
QIVLSQSPAILSASPGEKVTMTCRASSSVSYIHWFQQKPGSSPKPWIYATSNLASGVPVRFSGSGSGTSYSLTISRVEAEDAATYYCQQWTSNPPTFGGGTKLEIKRTVAAPSVFIFPPSDEQLKSGTASVVCLLNNFYPREAKVQWKVDNALQSGNSQESVTEQDSKDSTYSLSSTLTLSKADYEKHKVYACEVTHQGLSSPVTKSFNRGEC

SEQ ID NO: 31 - protein, 450 aa, synthetic construct
EVQLVESGGGLVQPGGSLRLSCAASGFNIKDTYIHWVRQAPGKGLEWVARIYPTNGYTRYADSVKGRFTISADTSKNTAYLQMNSLRAEDTAVYYCSRWGGDGFYAMDYWGQGTLVTVSSASTKGPSVFPLAPSSKSTSGGTAALGCLVKDYFPEPVTVSWNSGALTSGVHTFPAVLQSSGLYSLSSVVTVPSSSLGTQTYICNVNHKPSNTKVDKKVEPKSCDKTHTCPPCPAPELLGGPSVFLFPPKPKDTLMISRTPEVTCVVVDVSHEDPEVKFNWYVDGVEVHNAKTKPREEQYNSTYRVVSVLTVLHQDWLNGKEYKCKVSNKALPAPIEKTISKAKGQPREPQVYTLPPSRDELTKNQVSLTCLVKGFYPSDIAVEWESNGQPENNYKTTPPVLDSDGSFFLYSKLTVDKSRWQQGNVFSCSVMHEALHNHYTQKSLSLSPGK

SEQ ID NO: 32 - protein, 214 aa, synthetic construct
DIQMTQSPSSLSASVGDRVTITCRASQDVNTAVAWYQQKPGKAPKLLIYSASFLYSGVPSRFSGSRSGTDFTLTISSLQPEDFATYYCQQHYTTPPTFGQGTKVEIKRTVAAPSVFIFPPSDEQLKSGTASVVCLLNNFYPREAKVQWKVDNALQSGNSQESVTEQDSKDSTYSLSSTLTLSKADYEKHKVYACEVTHQGLSSPVTKSFNRGEC

SEQ ID NO: 33 - protein, 450 aa, synthetic construct
EVQLVESGGGLVQPGGSLRLSCAASGFNIKDTYIHWVRQAPGKGLEWVARIYPTNGGTRYADSVKGRFTISADTSKNTAYLQMNSLRAEDTAVYYCSRWGGDGFGAMDYWGQGTLVTVSSASTKGPSVFPLAPSSKSTSGGTAALGCLVKDYFPEPVTVSWNSGALTSGVHTFPAVLQSSGLYSLSSVVTVPSSSLGTQTYICNVNHKPSNTKVDKKVEPKSCDKTHTCPPCPAPELLGGPSVFLFPPKPKDTLMISRTPEVTCVVVDVSHEDPEVKFNWYVDGVEVHNAKTKPREEQYNSTYRVVSVLTVLHQDWLNGKEYKCKVSNKALPAPIEKTISKAKGQPREPQVYTLPPSRDELTKNQVSLTCLVKGFYPSDIAVEWESNGQPENNYKTTPPVLDSDGSFFLYSKLTVDKSRWQQGNVFSCSVMHEALHNHYTQKSLSLSPGK

SEQ ID NO: 34 - protein, 214 aa, synthetic construct
DIQMTQSPSSLSASVGDRVTITCRASQDVGTAVAWYQQKPGKAPKLLIYSASGLYSGVPSRFSGSRSGTDFTLTISSLQPEDFATYYCQQHGTTPPTFGQGTKVEIKRTVAAPSVFIFPPSDEQLKSGTASVVCLLNNFYPREAKVQWKVDNALQSGNSQESVTEQDSKDSTYSLSSTLTLSKADYEKHKVYACEVTHQGLSSPVTKSFNRGEC

SEQ ID NO: 35 - protein, 450 aa, synthetic construct
EVQLVESGGGLVQPGGSLRLSCAASGFNIKDTGIHWVRQAPGKGLEWVAGIYPTNGGTGYADSVKGRFTISADTSKNTAYLQMNSLRAEDTAVYYCSRGGGDGFGAMDYWGQGTLVTVSSASTKGPSVFPLAPSSKSTSGGTAALGCLVKDYFPEPVTVSWNSGALTSGVHTFPAVLQSSGLYSLSSVVTVPSSSLGTQTYICNVNHKPSNTKVDKKVEPKSCDKTHTCPPCPAPELLGGPSVFLFPPKPKDTLMISRTPEVTCVVVDVSHEDPEVKFNWYVDGVEVHNAKTKPREEQYNSTYRVVSVLTVLHQDWLNGKEYKCKVSNKALPAPIEKTISKAKGQPREPQVYTLPPSRDELTKNQVSLTCLVKGFYPSDIAVEWESNGQPENNYKTTPPVLDSDGSFFLYSKLTVDKSRWQQGNVFSCSVMHEALHNHYTQKSLSLSPGK

SEQ ID NO: 36 - DNA, 1350 bp, synthetic construct
  source 1..1350: mol_type = other DNA
caagtgcagctccagcagcccggggctgaactggtcaagcctggagcctcagtgaagatgtcctgcaaagcctccggctacacctttacatcttacaacatgcactgggtcaagcagaccccaggacggggcttggaatggattggtgccatctacccgggaaacggcgacactagctataaccagaagttcaagggcaaagcaaccctcaccgccgataagagcagcagcactgcgtacatgcagctgtcgtccctgacgtccgaggattccgccgtgtattactgcgcaaggtcaacctactatggaggagattggtacttcaacgtctggggagccgggaccactgtgactgtgtccgccgcgtcaactaagggcccttcagtgttccccctcgcgccaagctccaagtccactagcggcgggaccgccgcgctgggttgcctggtcaaggactacttccccgagcccgtgaccgtgtcctggaactccggcgcgctgacctccggggtgcatactttcccggctgtgcttcaatcgagcggactgtactccctgagctccgtggtcacggtgccgtcctcgagcctgggaacccagacctacatttgcaacgtgaaccacaagcccagcaacaccaaggtcgacaagaaggccgagcctaagtcctgtgacaagacccacacttgccctccgtgccccgcccctgagctgctgggagggccgtctgtgtttctcttcccgcccaagcctaaggacactctcatgatttcccgcacccccgaagtcacttgcgtggtggtggatgtgtcgcatgaagatccagaagtgaaattcaattggtacgtggatggagtggaagtgcacaacgccaagaccaaaccgcgcgaggagcagtacaattcaacctaccgggtggtgtcggtgttgactgtgctgcaccaggactggctgaacggaaaggagtacaagtgcaaagtgtcgaacaaggccctccctgctccgatcgaaaagaccatcagcaaggccaagggacagccgagggagccccaggtctacactctgcctccgtcccgcgacgagctgaccaagaaccaagtgtccctcacctgtcttgtgaaggggttctacccaagcgacatcgcggtcgaatgggaatcaaatggccagcctgagaacaactacaagacaacgcccccggtgctggactcggacggctcgttcttcctgtactccaagctgactgtggacaagtcccggtggcaacagggaaacgtgttcagctgtagcgtgatgcatgaagccctgcacaaccactacacccagaagtcgctctccctgtcacccggc

SEQ ID NO: 37 - DNA, 639 bp, synthetic construct
  source 1..639: mol_type = other DNA
cagatcgtgttgtcgcaatccccggccatcctgtccgcttcgccgggagaaaaggtcaccatgacttgtcgcgcctcaagcagcgtgtcctacattcattggtttcagcagaagcccgggtccagcccgaagccttggatctacgcaactagcaacctcgcctccggcgtgccagtgcgcttctccggttccggatcgggaacgtcctatagcctgactatctcgagagtggaggccgaggacgctgccacttactactgccagcagtggacctcgaatcctccaactttcggtggcggcaccaagctggagattaagaggaccgtcgcggcccctagcgtgttcattttccccccgtccgacgagcagctgaagtccgggacagcctcagtggtctgcctgctcaacaacttctacccccgggaagccaaagtgcagtggaaagtggataacgcgcttcagagcggcaactcacaagagtccgtgaccgaacaggactcgaaggacagcacctacagcctctcctccaccctgaccctgtcaaaggcggattacgaaaagcacaaggtctacgcctgcgaagtgacccaccaggggctgtcctctcccgtgaccaagtccttcaaccggggagagtgc

SEQ ID NO: 38 - DNA, 1350 bp, synthetic construct
  source 1..1350: mol_type = other DNA
gaagtccagctggtggaaagtggcggtggactggttcaaccaggaggaagcctaagactaagctgcgccgccagcggttttaacatcaaggacacatacatccattgggtccggcaggcacccggcaaaggtttagagtgggtcgcaaggatctaccccactaatggttataccaggtacgctgacagcgtgaagggcaggttcaccattagcgctgacaccagcaagaacactgcttatctgcagatgaatagcctgcgtgccgaagacacagccgtctattactgtagtagatggggaggtgatgggttctatgcgatggattactggggacagggcacactcgtgaccgttagtagcgctagcaccaagggcccatcggtcttccccctggcaccctcctccaagagcacctctgggggcacagcggccctgggctgcctggtcaaggactacttccccgaaccggtgacggtgtcgtggaactcaggcgccctgaccagcggcgtgcacaccttcccggctgtcctacagtcctcaggactctactccctcagcagcgtggtgaccgtgccctccagcagcttgggcacccagacctacatctgcaacgtgaatcacaagcccagcaacaccaaggtggacaagaaagtagagcccaaatcttgtgacaaaactcacacatgcccaccgtgcccagcacctgaactcctggggggaccgtcagtcttcctcttccccccaaaacccaaggacaccctcatgatctcccggacccctgaggtcacatgcgtggtggtggacgtgagccacgaagaccctgaggtcaagttcaactggtacgtggacggcgtggaggtgcataatgccaagacaaagccgcgggaggagcagtacaacagcacgtaccgtgtggtcagcgtcctcaccgtcctgcaccaggactggctgaatggcaaggagtacaagtgcaaggtctccaacaaagccctcccagcccccatcgagaaaaccatctccaaagccaaagggcagccccgagaaccacaggtgtacaccctgcccccatcccgggatgagctgaccaagaaccaggtcagcctgacctgcctggtcaaaggcttctatcccagcgacatcgccgtggagtgggagagcaatgggcagccggagaacaactacaagaccacgcctcccgtgctggactccgacggctccttcttcctctacagcaagctcaccgtggacaagagcaggtggcagcaggggaacgtcttctcatgctccgtgatgcatgaggctctgcacaaccactacacgcagaagagcctctccctgtctccgggtaaa

SEQ ID NO: 39 - DNA, 642 bp, synthetic construct
  source 1..642: mol_type = other DNA
gatatacagatgacgcagagccctagcagtctaagtgcaagcgttggagaccgtgtcaccattacctgccgcgctagccaggatgtcaacaccgcagtcgcctggtatcagcaaaaaccgggtaaggctccaaagctgttgatctacagtgccagctttctgtacagcggtgtgccaagtaggttcagcgggagccggagtgggacagactttacactcactattagcagtctgcagcccgaggacttcgccacctactactgtcagcagcattatacaacacccccaacattcgggcagggaaccaaagttgagataaaacgaacggttgccgcgccaagcgtatttatctttccccccagtgatgagcaactgaagagtggtacagccagcgttgtctgccttttgaataacttctatcctcgggaggcaaaggtccagtggaaagtggataatgcactccaaagcggtaacagccaggagagtgtgacagaacaggacagcaaagatagtacctacagcctcagtagtaccctcacactgagcaaagcggactatgaaaagcacaaggtgtacgcttgtgaagtgacccaccagggcctaagcagccctgttactaagagcttcaacagaggcgaatgt

SEQ ID NO: 40 - DNA, 1350 bp, synthetic construct
  source 1..1350: mol_type = other DNA
gaagtccagctggtggaaagtggcggtggactggttcaaccaggaggaagcctaagactaagctgcgccgccagcggttttaacatcaaggacacatacatccattgggtccggcaggcacccggcaaaggtttagagtgggtcgcaaggatctaccccactaatggtggcaccaggtacgctgacagcgtgaagggcaggttcaccattagcgctgacaccagcaagaacactgcttatctgcagatgaatagcctgcgtgccgaagacacagccgtctattactgtagtagatggggaggtgatgggttcggcgcgatggattactggggacagggcacactcgtgaccgttagtagcgctagcaccaagggcccatcggtcttccccctggcaccctcctccaagagcacctctgggggcacagcggccctgggctgcctggtcaaggactacttccccgaaccggtgacggtgtcgtggaactcaggcgccctgaccagcggcgtgcacaccttcccggctgtcctacagtcctcaggactctactccctcagcagcgtggtgaccgtgccctccagcagcttgggcacccagacctacatctgcaacgtgaatcacaagcccagcaacaccaaggtggacaagaaagtagagcccaaatcttgtgacaaaactcacacatgcccaccgtgcccagcacctgaactcctggggggaccgtcagtcttcctcttccccccaaaacccaaggacaccctcatgatctcccggacccctgaggtcacatgcgtggtggtggacgtgagccacgaagaccctgaggtcaagttcaactggtacgtggacggcgtggaggtgcataatgccaagacaaagccgcgggaggagcagtacaacagcacgtaccgtgtggtcagcgtcctcaccgtcctgcaccaggactggctgaatggcaaggagtacaagtgcaaggtctccaacaaagccctcccagcccccatcgagaaaaccatctccaaagccaaagggcagccccgagaaccacaggtgtacaccctgcccccatcccgggatgagctgaccaagaaccaggtcagcctgacctgcctggtcaaaggcttctatcccagcgacatcgccgtggagtgggagagcaatgggcagccggagaacaactacaagaccacgcctcccgtgctggactccgacggctccttcttcctctacagcaagctcaccgtggacaagagcaggtggcagcaggggaacgtcttctcatgctccgtgatgcatgaggctctgcacaaccactacacgcagaagagcctctccctgtctccgggtaaa

SEQ ID NO: 41 - DNA, 642 bp, synthetic construct
  source 1..642: mol_type = other DNA
gatatacagatgacgcagagccctagcagtctaagtgcaagcgttggagaccgtgtcaccattacctgccgcgctagccaggatgtcggcaccgcagtcgcctggtatcagcaaaaaccgggtaaggctccaaagctgttgatctacagtgccagcggcctgtacagcggtgtgccaagtaggttcagcgggagccggagtgggacagactttacactcactattagcagtctgcagcccgaggacttcgccacctactactgtcagcagcatggcacaacacccccaacattcgggcagggaaccaaagttgagataaaacgaacggttgccgcgccaagcgtatttatctttccccccagtgatgagcaactgaagagtggtacagccagcgttgtctgccttttgaataacttctatcctcgggaggcaaaggtccagtggaaagtggataatgcactccaaagcggtaacagccaggagagtgtgacagaacaggacagcaaagatagtacctacagcctcagtagtaccctcacactgagcaaagcggactatgaaaagcacaaggtgtacgcttgtgaagtgacccaccagggcctaagcagccctgttactaagagcttcaacagaggcgaatgt

SEQ ID NO: 42 - DNA, 1350 bp, synthetic construct
  source 1..1350: mol_type = other DNA
gaagtccagctggtggaaagtggcggtggactggttcaaccaggaggaagcctaagactaagctgcgccgccagcggttttaacatcaaggacacaggcatccattgggtccggcaggcacccggcaaaggtttagagtgggtcgcaggcatctaccccactaatggtggcaccggctacgctgacagcgtgaagggcaggttcaccattagcgctgacaccagcaagaacactgcttatctgcagatgaatagcctgcgtgccgaagacacagccgtctattactgtagtagaggcggaggtgatgggttcggcgcgatggattactggggacagggcacactcgtgaccgttagtagcgctagcaccaagggcccatcggtcttccccctggcaccctcctccaagagcacctctgggggcacagcggccctgggctgcctggtcaaggactacttccccgaaccggtgacggtgtcgtggaactcaggcgccctgaccagcggcgtgcacaccttcccggctgtcctacagtcctcaggactctactccctcagcagcgtggtgaccgtgccctccagcagcttgggcacccagacctacatctgcaacgtgaatcacaagcccagcaacaccaaggtggacaagaaagtagagcccaaatcttgtgacaaaactcacacatgcccaccgtgcccagcacctgaactcctggggggaccgtcagtcttcctcttccccccaaaacccaaggacaccctcatgatctcccggacccctgaggtcacatgcgtggtggtggacgtgagccacgaagaccctgaggtcaagttcaactggtacgtggacggcgtggaggtgcataatgccaagacaaagccgcgggaggagcagtacaacagcacgtaccgtgtggtcagcgtcctcaccgtcctgcaccaggactggctgaatggcaaggagtacaagtgcaaggtctccaacaaagccctcccagcccccatcgagaaaaccatctccaaagccaaagggcagccccgagaaccacaggtgtacaccctgcccccatcccgggatgagctgaccaagaaccaggtcagcctgacctgcctggtcaaaggcttctatcccagcgacatcgccgtggagtgggagagcaatgggcagccggagaacaactacaagaccacgcctcccgtgctggactccgacggctccttcttcctctacagcaagctcaccgtggacaagagcaggtggcagcaggggaacgtcttctcatgctccgtgatgcatgaggctctgcacaaccactacacgcagaagagcctctccctgtctccgggtaaa

SEQ ID NO: 43 - DNA, 20 bp, synthetic construct
  source 1..20: mol_type = other DNA
cctctagagtccggaggctg

SEQ ID NO: 44 - DNA, 26 bp, synthetic construct
  source 1..26: mol_type = other DNA
ccctaccggttagtaatgagtttgat

SEQ ID NO: 45 - DNA, 37 bp, synthetic construct
  source 1..37: mol_type = other DNA
gcctccggactctagagggccaccatgggttggtccc

SEQ ID NO: 46 - DNA, 39 bp, synthetic construct
  source 1..39: mol_type = other DNA
cattactaaccggtagggtcagccgggtgacagggagag

SEQ ID NO: 47 - DNA, 39 bp, synthetic construct
  source 1..39: mol_type = other DNA
gcctccggactctagagggccaccatggacttccaagtg

SEQ ID NO: 48 - DNA, 39 bp, synthetic construct
  source 1..39: mol_type = other DNA
cattactaaccggtagggtcagcactctccccggttgaa

SEQ ID NO: 49 - DNA, 38 bp, synthetic construct
  source 1..38: mol_type = other DNA
gcctccggactctagagggccaccatgagtgtgcccac

SEQ ID NO: 50 - DNA, 44 bp, synthetic construct
  source 1..44: mol_type = other DNA
cattactaaccggtagggtctcatttacccggagacagggagag

SEQ ID NO: 51 - DNA, 38 bp, synthetic construct
  source 1..38: mol_type = other DNA
gcctccggactctagagggccaccatggaatggagctg

SEQ ID NO: 52 - DNA, 43 bp, synthetic construct
  source 1..43: mol_type = other DNA
cattactaaccggtagggtcaacattcgcctctgttgaagctc

SEQ ID NO: 53 - DNA, 38 bp, synthetic construct; identical to SEQ ID NO: 49
  source 1..38: mol_type = other DNA

SEQ ID NO: 54 - DNA, 42 bp, synthetic construct
  source 1..42: mol_type = other DNA
cattactaaccggtagggtcatttacccggagacagggagag

SEQ ID NO: 55 - DNA, 38 bp, synthetic construct; identical to SEQ ID NO: 51
  source 1..38: mol_type = other DNA

SEQ ID NO: 56 - DNA, 43 bp, synthetic construct; identical to SEQ ID NO: 52
  source 1..43: mol_type = other DNA

SEQ ID NO: 57 - protein, 807 aa, synthetic construct
EGVAAALTPERLLEWQDKGIFVIQSESLKKCIQAGKSVLTLENCKQANKHMLWKWVSNHGLFNIGGSGCLGLNFSAPEQPLSLYECDSTLVSLRWRCNRKMITGPLQYSVQVAHDNTVVASRKYIHKWISYGSGGGDICEYLHKDLHTIKGNTHGMPCMFPFQYNHQWHHECTREGREDDLLWCATTSRYERDEKWGFCPDPTSAEVGCDTIWEKDLNSHICYQFNLLSSLSWSEAHSSCQMQGGTLLSITDETEENFIREHMSSKTVEVWMGLNQLDEHAGWQWSDGTPLNYLNWSPEVNFEPFVEDHCGTFSSFMPSAWRSRDCESTLPYICKKYLNHIDHEIVEGGGGSGGGGSEVQLVESGGGLVQPGGSLRLSCAASGFNIGGTGIHWVRQAPGKGLEWVAGIYPTNGGTGYAGSVKGRFTISADTSKNTAYLQMNSLRAEDTAVYYCSRGGGDGFGAMGYWGQGTLVTVSSASTKGPSVFPLAPSSKSTSGGTAALGCLVKDYFPEPVTVSWNSGALTSGVHTFPAVLQSSGLYSLSSVVTVPSSSLGTQTYICNVNHKPSNTKVDKKVEPKSCDKTHTCPPCPAPELLGGPSVFLFPPKPKDTLMISRTPEVTCVVVDVSHEDPEVKFNWYVDGVEVHNAKTKPREEQYNSTYRVVSVLTVLHQDWLNGKEYKCKVSNKALPAPIEKTISKAKGQPREPQVYTLPPSRDELTKNQVSLTCLVKGFYPSDIAVEWESNGQPENNYKTTPPVLDSDGSFFLYSKLTVDKSRWQQGNVFSCSVMHEALHNHYTQKSLSLSPGK

SEQ ID NO: 58 - DNA, 2421 bp, synthetic construct
  source 1..2421: mol_type = other DNA
gagggtgtggcggcggcgcttacccccgagcggctcctggagtggcaggataaaggaatatttgttatccaaagtgagagtctcaagaaatgcattcaagcaggtaaatcggttctgaccctggagaactgcaagcaagcaaacaagcacatgctgtggaaatgggtttcaaaccatggcctctttaacataggaggcagtggttgcctgggcctgaatttctccgccccagagcagccattaagcttatatgaatgtgactccaccctcgtttccttacggtggcgctgtaacaggaagatgatcacaggcccgctgcagtactctgtccaggtggcgcatgacaacacagtggtggcctcacggaagtatattcataagtggatttcttatgggtcaggtggtggagacatttgtgaatatctacacaaagatttgcatacaatcaaagggaacacccacgggatgccgtgtatgtttcccttccagtataaccatcagtggcatcatgaatgtacccgtgaaggtcgggaagatgacttactgtggtgtgccacgacaagccgttatgaaagagatgaaaagtggggattttgccctgatcccacctctgcagaagtaggttgtgatactatttgggagaaggacctcaattcacacatttgctaccagttcaacctgctttcatctctctcttggagtgaggcacattcttcatgccagatgcaaggaggtacgctgttaagtattacagatgaaactgaagaaaatttcataagggagcacatgagcagtaaaacagtggaggtgtggatgggcctcaatcagctggatgaacacgctggctggcagtggtctgatggaacgccgctcaactatctgaattggagcccagaggtaaattttgagccatttgttgaagatcactgtggaacatttagttcatttatgccaagtgcctggaggagtcgggattgtgagtccaccttgccatatatatgtaaaaaatatctaaaccacattgatcatgaaatagttgaaggcggtggaggctccggcggaggtggaagcgaagtccagctggtggaaagtggcggtggactggttcaaccaggaggaagcctaagactaagctgcgccgccagcggttttaacatcggtggcacaggcatccattgggtccggcaggcacccggcaaaggtttagagtgggtcgcaggcatctaccccactaatggtggcaccggctacgctggtagcgtgaagggcaggttcaccattagcgctgacaccagcaagaacactgcttatctgcagatgaatagcctgcgtgccgaagacacagccgtctattactgtagtagaggcggaggtgatgggttcggcgcgatgggctactggggacagggcacactcgtgaccgttagtagcgctagcaccaagggcccatcggtcttccccctggcaccctcctccaagagcacctctgggggcacagcggccctgggctgcctggtcaaggactacttccccgaaccggtgacggtgtcgtggaactcaggcgccctgaccagcggcgtgcacaccttcccggctgtcctacagtcctcaggactctactccctcagcagcgtggtgaccgtgccctccagcagcttgggcacccagacctacatctgcaacgtgaatcacaagcccagcaacaccaaggtggacaagaaagtagagcccaaatcttgtgacaaaactcacacatgcccaccgtgcccagcacctgaactcctggggggaccgtcagtcttcctcttccccccaaaacccaaggacaccctcatgatctcccggacccctgaggtcacatgcgtggtggtggacgtgagccacgaagaccctgaggtcaagttcaactggtacgtggacggcgtggaggtgcataatgccaagacaaagccgcgggaggagcagtacaacagcacgtaccgtgtggtcagcgtcctcaccgtcctgcaccaggactggctgaatggcaaggagtacaagtgcaaggtctccaacaaagccctcccagcccccatcgagaaaaccatctccaaagccaaagggcagccccgagaaccacaggtgtacaccctgcccccatcccgggatgagctgaccaagaaccaggtcagcctgacctgcctggtcaaaggcttctatcccagcgacatcgccgtggagtgggagagcaatgggcagccggagaacaactacaagaccacgcctcccgtgctggactccgacggctccttcttcctctacagcaagctcaccgtggacaagagcaggtggcagcaggggaacgtcttctcatgctccgtgatgcatgaggctctgcacaaccactacacgcagaagagcctctccctgtctccgggtaaa

SEQ ID NO: 59 - protein, 571 aa, synthetic construct
EGVAAALTPERLLEWQDKGIFVIQSESLKKCIQAGKSVLTLENCKQANKHMLWKWVSNHGLFNIGGSGCLGLNFSAPEQPLSLYECDSTLVSLRWRCNRKMITGPLQYSVQVAHDNTVVASRKYIHKWISYGSGGGDICEYLHKDLHTIKGNTHGMPCMFPFQYNHQWHHECTREGREDDLLWCATTSRYERDEKWGFCPDPTSAEVGCDTIWEKDLNSHICYQFNLLSSLSWSEAHSSCQMQGGTLLSITDETEENFIREHMSSKTVEVWMGLNQLDEHAGWQWSDGTPLNYLNWSPEVNFEPFVEDHCGTFSSFMPSAWRSRDCESTLPYICKKYLNHIDHEIVEGGGGSGGGGSDIQMTQSPSSLSASVGDRVTITCRASQGVGTAVAWYQQKPGKAPKLLIYSASGLYSGVPSRFSGSRSGTDFTLTISSLQPEDFATYYCQQHGTTPPTFGQGTKVEIKRTVAAPSVFIFPPSDEQLKSGTASVVCLLNNFYPREAKVQWKVDNALQSGNSQESVTEQDSKDSTYSLSSTLTLSKADYEKHKVYACEVTHQGLSSPVTKSFNRGEC

SEQ ID NO: 60 - DNA, 1713 bp, synthetic construct
  source 1..1713: mol_type = other DNA
gagggtgtggcggcggcgcttacccccgagcggctcctggagtggcaggataaaggaatatttgttatccaaagtgagagtctcaagaaatgcattcaagcaggtaaatcggttctgaccctggagaactgcaagcaagcaaacaagcacatgctgtggaaatgggtttcaaaccatggcctctttaacataggaggcagtggttgcctgggcctgaatttctccgccccagagcagccattaagcttatatgaatgtgactccaccctcgtttccttacggtggcgctgtaacaggaagatgatcacaggcccgctgcagtactctgtccaggtggcgcatgacaacacagtggtggcctcacggaagtatattcataagtggatttcttatgggtcaggtggtggagacatttgtgaatatctacacaaagatttgcatacaatcaaagggaacacccacgggatgccgtgtatgtttcccttccagtataaccatcagtggcatcatgaatgtacccgtgaaggtcgggaagatgacttactgtggtgtgccacgacaagccgttatgaaagagatgaaaagtggggattttgccctgatcccacctctgcagaagtaggttgtgatactatttgggagaaggacctcaattcacacatttgctaccagttcaacctgctttcatctctctcttggagtgaggcacattcttcatgccagatgcaaggaggtacgctgttaagtattacagatgaaactgaagaaaatttcataagggagcacatgagcagtaaaacagtggaggtgtggatgggcctcaatcagctggatgaacacgctggctggcagtggtctgatggaacgccgctcaactatctgaattggagcccagaggtaaattttgagccatttgttgaagatcactgtggaacatttagttcatttatgccaagtgcctggaggagtcgggattgtgagtccaccttgccatatatatgtaaaaaatatctaaaccacattgatcatgaaatagttgaaggcggtggaggctccggcggaggtggaagcgatatacagatgacgcagagccctagcagtctaagtgcaagcgttggagaccgtgtcaccattacctgccgcgctagccagggcgtcggcaccgcagtcgcctggtatcagcaaaaaccgggtaaggctccaaagctgttgatctacagtgccagcggcctgtacagcggtgtgccaagtaggttcagcgggagccggagtgggacagactttacactcactattagcagtctgcagcccgaggacttcgccacctactactgtcagcagcatggcacaacacccccaacattcgggcagggaaccaaagttgagataaaacgaacggttgccgcgccaagcgtatttatctttccccccagtgatgagcaactgaagagtggtacagccagcgttgtctgccttttgaataacttctatcctcgggaggcaaaggtccagtggaaagtggataatgcactccaaagcggtaacagccaggagagtgtgacagaacaggacagcaaagatagtacctacagcctcagtagtaccctcacactgagcaaagcggactatgaaaagcacaaggtgtacgcttgtgaagtgacccaccagggcctaagcagccctgttactaagagcttcaacagaggcgaatgt

SEQ ID NO: 61 - protein, 582 aa, synthetic construct
EGVAAALTPERLLEWQDKGIFVIQSESLKKCIQAGKSVLTLENCKQANKHMLWKWVSNHGLFNIGGSGCLGLNFSAPEQPLSLYECDSTLVSLRWRCNRKMITGPLQYSVQVAHDNTVVASRKYIHKWISYGSGGGDICEYLHKDLHTIKGNTHGMPCMFPFQYNHQWHHECTREGREDDLLWCATTSRYERDEKWGFCPDPTSAEVGCDTIWEKDLNSHICYQFNLLSSLSWSEAHSSCQMQGGTLLSITDETEENFIREHMSSKTVEVWMGLNQLDEHAGWQWSDGTPLNYLNWSPEVNFEPFVEDHCGTFSSFMPSAWRSRDCESTLPYICKKYLNHIDHEIVEGGGGSGGGGSTHTCPPCPAPELLGGPSVFLFPPKPKDTLMISRTPEVTCVVVDVSHEDPEVKFNWYVDGVEVHNAKTKPREEQYNSTYRVVSVLTVLHQDWLNGKEYKCKVSNKALPAPIEKTISKAKGQPREPQVYTLPPSRDELTKNQVSLTCLVKGFYPSDIAVEWESNGQPENNYKTTPPVLDSDGSFFLYSKLTVDKSRWQQGNVFSCSVMHEALHNHYTQKSLSLSPGK

SEQ ID NO: 62 - DNA, 1746 bp, synthetic construct
  source 1..1746: mol_type = other DNA
gagggtgtggcggcggcgcttacccccgagcggctcctggagtggcaggataaaggaatatttgttatccaaagtgagagtctcaagaaatgcattcaagcaggtaaatcggttctgaccctggagaactgcaagcaagcaaacaagcacatgctgtggaaatgggtttcaaaccatggcctctttaacataggaggcagtggttgcctgggcctgaatttctccgccccagagcagccattaagcttatatgaatgtgactccaccctcgtttccttacggtggcgctgtaacaggaagatgatcacaggcccgctgcagtactctgtccaggtggcgcatgacaacacagtggtggcctcacggaagtatattcataagtggatttcttatgggtcaggtggtggagacatttgtgaatatctacacaaagatttgcatacaatcaaagggaacacccacgggatgccgtgtatgtttcccttccagtataaccatcagtggcatcatgaatgtacccgtgaaggtcgggaagatgacttactgtggtgtgccacgacaagccgttatgaaagagatgaaaagtggggattttgccctgatcccacctctgcagaagtaggttgtgatactatttgggagaaggacctcaattcacacatttgctaccagttcaacctgctttcatctctctcttggagtgaggcacattcttcatgccagatgcaaggaggtacgctgttaagtattacagatgaaactgaagaaaatttcataagggagcacatgagcagtaaaacagtggaggtgtggatgggcctcaatcagctggatgaacacgctggctggcagtggtctgatggaacgccgctcaactatctgaattggagcccagaggtaaattttgagccatttgttgaagatcactgtggaacatttagttcatttatgccaagtgcctggaggagtcgggattgtgagtccaccttgccatatatatgtaaaaaatatctaaaccacattgatcatgaaatagttgaaggcggtggaggctccggcggaggtggaagcactcacacatgcccaccgtgcccagcacctgaactcctggggggaccgtcagtcttcctcttccccccaaaacccaaggacaccctcatgatctcccggacccctgaggtcacatgcgtggtggtggacgtgagccacgaagaccctgaggtcaagttcaactggtacgtggacggcgtggaggtgcataatgccaagacaaagccgcgggaggagcagtacaacagcacgtaccgtgtggtcagcgtcctcaccgtcctgcaccaggactggctgaatggcaaggagtacaagtgcaaggtctccaacaaagccctcccagcccccatcgagaaaaccatctccaaagccaaagggcagccccgagaaccacaggtgtacaccctgcccccatcccgggatgagctgaccaagaaccaggtcagcctgacctgcctggtcaaaggcttctatcccagcgacatcgccgtggagtgggagagcaatgggcagccggagaacaactacaagaccacgcctcccgtgctggactccgacggctccttcttcctctacagcaagctcaccgtggacaagagcaggtggcagcaggggaacgtcttctcatgctccgtgatgcatgaggctctgcacaaccactacacgcagaagagcctctccctgtctccgggtaaa

SEQ ID NO: 63 - protein, 950 aa, synthetic construct
EGVAAALTPERLLEWQDKGIFVIQSESLKKCIQAGKSVLTLENCKQANKHMLWKWVSNHGLFNIGGSGCLGLNFSAPEQPLSLYECDSTLVSLRWRCNRKMITGPLQYSVQVAHDNTVVASRKYIHKWISYGSGGGDICEYLHKDLHTIKGNTHGMPCMFPFQYNHQWHHECTREGREDDLLWCATTSRYERDEKWGFCPDPTSAEVGCDTIWEKDLNSHICYQFNLLSSLSWSEAHSSCQMQGGTLLSITDETEENFIREHMSSKTVEVWMGLNQLDEHAGWQWSDGTPLNYLNWSPEVNFEPFVEDHCGTFSSFMPSAWRSRDCESTLPYICKKYLNHIDHEIVEKDAWKYYATHCEPGWNPYNRNCYKLQKEEKTWHEALRSCQADNSALIDITSLAEVEFLVTLLGDENASETWIGLSSNKIPVSFEWSNDSSVIFTNWHTLEPHIFPNRSQLCVSAEQSEGHWKVKNCEERLFYICKKAGHVLSDGGGGSGGGGSEVQLVESGGGLVQPGGSLRLSCAASGFNIGGTGIHWVRQAPGKGLEWVAGIYPTNGGTGYAGSVKGRFTISADTSKNTAYLQMNSLRAEDTAVYYCSRGGGDGFGAMGYWGQGTLVTVSSASTKGPSVFPLAPSSKSTSGGTAALGCLVKDYFPEPVTVSWNSGALTSGVHTFPAVLQSSGLYSLSSVVTVPSSSLGTQTYICNVNHKPSNTKVDKKVEPKSCDKTHTCPPCPAPELLGGPSVFLFPPKPKDTLMISRTPEVTCVVVDVSHEDPEVKFNWYVDGVEVHNAKTKPREEQYNSTYRVVSVLTVLHQDWLNGKEYKCKVSNKALPAPIEKTISKAKGQPREPQVYTLPPSRDELTKNQVSLTCLVKGFYPSDIAVEWESNGQPENNYKTTPPVLDSDGSFFLYSKLTVDKSRWQQGNVFSCSVMHEALHNHYTQKSLSLSPGK

SEQ ID NO: 64 - DNA, 2850 bp, synthetic construct
  source 1..2850: mol_type = other DNA
gagggtgtggcggcggcgcttacccccgagcggctcctggagtggcaggataaaggaatatttgttatccaaagtgagagtctcaagaaatgcattcaagcaggtaaatcggttctgaccctggagaactgcaagcaagcaaacaagcacatgctgtggaaatgggtttcaaaccatggcctctttaacataggaggcagtggttgcctgggcctgaatttctccgccccagagcagccattaagcttatatgaatgtgactccaccctcgtttccttacggtggcgctgtaacaggaagatgatcacaggcccgctgcagtactctgtccaggtggcgcatgacaacacagtggtggcctcacggaagtatattcataagtggatttcttatgggtcaggtggtggagacatttgtgaatatctacacaaagatttgcatacaatcaaagggaacacccacgggatgccgtgtatgtttcccttccagtataaccatcagtggcatcatgaatgtacccgtgaaggtcgggaagatgacttactgtggtgtgccacgacaagccgttatgaaagagatgaaaagtggggattttgccctgatcccacctctgcagaagtaggttgtgatactatttgggagaaggacctcaattcacacatttgctaccagttcaacctgctttcatctctctcttggagtgaggcacattcttcatgccagatgcaaggaggtacgctgttaagtattacagatgaaactgaagaaaatttcataagggagcacatgagcagtaaaacagtggaggtgtggatgggcctcaatcagctggatgaacacgctggctggcagtggtctgatggaacgccgctcaactatctgaattggagcccagaggtaaattttgagccatttgttgaagatcactgtggaacatttagttcatttatgccaagtgcctggaggagtcgggattgtgagtccaccttgccatatatatgtaaaaaatatctaaaccacattgatcatgaaatagttgaaaaagatgcgtggaaatattatgctacccactgtgagcctggctggaatccctacaatcgtaattgctacaaacttcagaaagaagaaaagacctggcatgaggctctgcgttcttgtcaggctgataacagtgcattaatagacataacctcattagcagaggtggagtttcttgtaaccctccttggagatgaaaatgcatcagaaacatggattggtttgagcagcaataaaattccagtttcctttgaatggtctaatgactcttcagtcatctttactaattggcacacacttgagccccacatttttccaaatagaagccagctgtgtgtctcagcagagcagtctgagggacactggaaagtcaaaaattgtgaagaaagacttttttacatttgtaaaaaagcaggccatgtcctctctgatggcggtggaggctccggcggaggtggaagcgaagtccagctggtggaaagtggcggtggactggttcaaccaggaggaagcctaagactaagctgcgccgccagcggttttaacatcggtggcacaggcatccattgggtccggcaggcacccggcaaaggtttagagtgggtcgcaggcatctaccccactaatggtggcaccggctacgctggtagcgtgaagggcaggttcaccattagcgctgacaccagcaagaacactgcttatctgcagatgaatagcctgcgtgccgaagacacagccgtctattactgtagtagaggcggaggtgatgggttcggcgcgatgggctactggggacagggcacactcgtgaccgttagtagcgctagcaccaagggcccatcggtcttccccctggcaccctcctccaagagcacctctgggggcacagcggccctgggctgcctggtcaaggactacttccccgaaccggtgacggtgtcgtggaactcaggcgccctgaccagcggcgtgcacaccttcccggctgtcctacagtcctcaggactctactccctcagcagcgtggtgaccgtgccctccagcagcttgggcacccagacctacatctgcaacgtgaatcacaagcccagcaacaccaaggtggacaagaaagtagagcccaaatcttgtgacaaaactcacacatgcccaccgtgcccagcacctgaactcctggggggaccgtcagtcttcctcttccccccaaaacccaaggacaccctcatgatctcccggacccctgaggtcacatgcgtggtggtggacgtgagccacgaagaccctgaggtcaagttcaactggtacgtggacggcgtggaggtgcataatgccaagacaaagccgcgggaggagcagtacaacagcacgtaccgtgtggtcagcgtcctcaccgtcctgcaccaggactggctgaatggcaaggagtacaagtgcaaggtctccaacaaagccctcccagcccccatcgagaaaaccatctccaaagccaaagggcagccccgagaaccacaggtgtacaccctgcccccatcccgggatgagctgaccaagaaccaggtcagcctgacctgcctggtcaaaggcttctatcccagcgacatcgccgtggagtgggagagcaatgggcagccggagaacaactacaagaccacgcctcccgtgctggactccgacggctccttcttcctctacagcaagctcaccgtggacaagagcaggtggcagcaggggaacgtcttctcatgctccgtgatgcatgaggctctgcacaaccactacacgcagaagagcctctccctgtctccgggtaaa

SEQ ID NO: 65 - protein, 714 aa, synthetic construct
EGVAAALTPERLLEWQDKGIFVIQSESLKKCIQAGKSVLTLENCKQANKHMLWKWVSNHGLFNIGGSGCLGLNFSAPEQPLSLYECDSTLVSLRWRCNRKMITGPLQYSVQVAHDNTVVASRKYIHKWISYGSGGGDICEYLHKDLHTIKGNTHGMPCMFPFQYNHQWHHECTREGREDDLLWCATTSRYERDEKWGFCPDPTSAEVGCDTIWEKDLNSHICYQFNLLSSLSWSEAHSSCQMQGGTLLSITDETEENFIREHMSSKTVEVWMGLNQLDEHAGWQWSDGTPLNYLNWSPEVNFEPFVEDHCGTFSSFMPSAWRSRDCESTLPYICKKYLNHIDHEIVEKDAWKYYATHCEPGWNPYNRNCYKLQKEEKTWHEALRSCQADNSALIDITSLAEVEFLVTLLGDENASETWIGLSSNKIPVSFEWSNDSSVIFTNWHTLEPHIFPNRSQLCVSAEQSEGHWKVKNCEERLFYICKKAGHVLSDGGGGSGGGGSDIQMTQSPSSLSASVGDRVTITCRASQGVGTAVAWYQQKPGKAPKLLIYSASGLYSGVPSRFSGSRSGTDFTLTISSLQPEDFATYYCQQHGTTPPTFGQGTKVEIKRTVAAPSVFIFPPSDEQLKSGTASVVCLLNNFYPREAKVQWKVDNALQSGNSQESVTEQDSKDSTYSLSSTLTLSKADYEKHKVYACEVTHQGLSSPVTKSFNRGEC

SEQ ID NO: 66 - DNA, 2142 bp, synthetic construct
  source 1..2142: mol_type = other DNA
gagggtgtggcggcggcgcttacccccgagcggctcctggagtggcaggataaaggaatatttgttatccaaagtgagagtctcaagaaatgcattcaagcaggtaaatcggttctgaccctggagaactgcaagcaagcaaacaagcacatgctgtggaaatgggtttcaaaccatggcctctttaacataggaggcagtggttgcctgggcctgaatttctccgccccagagcagccattaagcttatatgaatgtgactccaccctcgtttccttacggtggcgctgtaacaggaagatgatcacaggcccgctgcagtactctgtccaggtggcgcatgacaacacagtggtggcctcacggaagtatattcataagtggatttcttatgggtcaggtggtggagacatttgtgaatatctacacaaagatttgcatacaatcaaagggaacacccacgggatgccgtgtatgtttcccttccagtataaccatcagtggcatcatgaatgtacccgtgaaggtcgggaagatgacttactgtggtgtgccacgacaagccgttatgaaagagatgaaaagtggggattttgccctgatcccacctctgcagaagtaggttgtgatactatttgggagaaggacctcaattcacacatttgctaccagttcaacctgctttcatctctctcttggagtgaggcacattcttcatgccagatgcaaggaggtacgctgttaagtattacagatgaaactgaagaaaatttcataagggagcacatgagcagtaaaacagtggaggtgtggatgggcctcaatcagctggatgaacacgctggctggcagtggtctgatggaacgccgctcaactatctgaattggagcccagaggtaaattttgagccatttgttgaagatcactgtggaacatttagttcatttatgccaagtgcctggaggagtcgggattgtgagtccaccttgccatatatatgtaaaaaatatctaaaccacattgatcatgaaatagttgaaaaagatgcgtggaaatattatgctacccactgtgagcctggctggaatccctacaatcgtaattgctacaaacttcagaaagaagaaaagacctggcatgaggctctgcgttcttgtcaggctgataacagtgcattaatagacataacctcattagcagaggtggagtttcttgtaaccctccttggagatgaaaatgcatcagaaacatggattggtttgagcagcaataaaattccagtttcctttgaatggtctaatgactcttcagtcatctttactaattggcacacacttgagccccacatttttccaaatagaagccagctgtgtgtctcagcagagcagtctgagggacactggaaagtcaaaaattgtgaagaaagacttttttacatttgtaaaaaagcaggccatgtcctctctgatggcggtggaggctccggcggaggtggaagcgatatacagatgacgcagagccctagcagtctaagtgcaagcgttggagaccgtgtcaccattacctgccgcgctagccagggcgtcggcaccgcagtcgcctggtatcagcaaaaaccgggtaaggctccaaagctgttgatctacagtgccagcggcctgtacagcggtgtgccaagtaggttcagcgggagccggagtgggacagactttacactcactattagcagtctgcagcccgaggacttcgccacctactactgtcagcagcatggcacaacacccccaacattcgggcagggaaccaaagttgagataaaacgaacggttgccgcgccaagcgtatttatctttccccccagtgatgagcaactgaagagtggtacagccagcgttgtctgccttttgaataacttctatcctcgggaggcaaaggtccagtggaaagtggataatgcactccaaagcggtaacagccaggagagtgtgacagaacaggacagcaaagatagtacctacagcctcagtagtaccctcacactgagcaaagcggactatgaaaagcacaaggtgtacgcttgtgaagtgacccaccagggcctaagcagccctgttactaagagcttcaacagaggcgaatgt

SEQ ID NO: 67 - protein, 725 aa, synthetic construct
EGVAAALTPERLLEWQDKGIFVIQSESLKKCIQAGKSVLTLENCKQANKHMLWKWVSNHGLFNIGGSGCLGLNFSAPEQPLSLYECDSTLVSLRWRCNRKMITGPLQYSVQVAHDNTVVASRKYIHKWISYGSGGGDICEYLHKDLHTIKGNTHGMPCMFPFQYNHQWHHECTREGREDDLLWCATTSRYERDEKWGFCPDPTSAEVGCDTIWEKDLNSHICYQFNLLSSLSWSEAHSSCQMQGGTLLSITDETEENFIREHMSSKTVEVWMGLNQLDEHAGWQWSDGTPLNYLNWSPEVNFEPFVEDHCGTFSSFMPSAWRSRDCESTLPYICKKYLNHIDHEIVEKDAWKYYATHCEPGWNPYNRNCYKLQKEEKTWHEALRSCQADNSALIDITSLAEVEFLVTLLGDENASETWIGLSSNKIPVSFEWSNDSSVIFTNWHTLEPHIFPNRSQLCVSAEQSEGHWKVKNCEERLFYICKKAGHVLSDGGGGSGGGGSTHTCPPCPAPELLGGPSVFLFPPKPKDTLMISRTPEVTCVVVDVSHEDPEVKFNWYVDGVEVHNAKTKPREEQYNSTYRVVSVLTVLHQDWLNGKEYKCKVSNKALPAPIEKTISKAKGQPREPQVYTLPPSRDELTKNQVSLTCLVKGFYPSDIAVEWESNGQPENNYKTTPPVLDSDGSFFLYSKLTVDKSRWQQGNVFSCSVMHEALHNHYTQKSLSLSPGK

SEQ ID NO: 68 - DNA, 2175 bp, synthetic construct
  source 1..2175: mol_type = other DNA
gagggtgtggcggcggcgcttacccccgagcggctcctggagtggcaggataaaggaatatttgttatccaaagtgagagtctcaagaaatgcattcaagcaggtaaatcggttctgaccctggagaactgcaagcaagcaaacaagcacatgctgtggaaatgggtttcaaaccatggcctctttaacataggaggcagtggttgcctgggcctgaatttctccgccccagagcagccattaagcttatatgaatgtgactccaccctcgtttccttacggtggcgctgtaacaggaagatgatcacaggcccgctgcagtactctgtccaggtggcgcatgacaacacagtggtggcctcacggaagtatattcataagtggatttcttatgggtcaggtggtggagacatttgtgaatatctacacaaagatttgcatacaatcaaagggaacacccacgggatgccgtgtatgtttcccttccagtataaccatcagtggcatcatgaatgtacccgtgaaggtcgggaagatgacttactgtggtgtgccacgacaagccgttatgaaagagatgaaaagtggggattttgccctgatcccacctctgcagaagtaggttgtgatactatttgggagaaggacctcaattcacacatttgctaccagttcaacctgctttcatctctctcttggagtgaggcacattcttcatgccagatgcaaggaggtacgctgttaagtattacagatgaaactgaagaaaatttcataagggagcacatgagcagtaaaacagtggaggtgtggatgggcctcaatcagctggatgaacacgctggctggcagtggtctgatggaacgccgctcaactatctgaattggagcccagaggtaaattttgagccatttgttgaagatcactgtggaacatttagttcatttatgccaagtgcctggaggagtcgggattgtgagtccaccttgccatatatatgtaaaaaatatctaaaccacattgatcatgaaatagttgaaaaagatgcgtggaaatattatgctacccactgtgagcctggctggaatccctacaatcgtaattgctacaaacttcagaaagaagaaaagacctggcatgaggctctgcgttcttgtcaggctgataacagtgcattaatagacataacctcattagcagaggtggagtttcttgtaaccctccttggagatgaaaatgcatcagaaacatggattggtttgagcagcaataaaattccagtttcctttgaatggtctaatgactcttcagtcatctttactaattggcacacacttgagccccacatttttccaaatagaagccagctgtgtgtctcagcagagcagtctgagggacactggaaagtcaaaaattgtgaagaaagacttttttacatttgtaaaaaagcaggccatgtcctctctgatggcggtggaggctccggcggaggtggaagcactcacacatgcccaccgtgcccagcacctgaactcctggggggaccgtcagtcttcctcttccccccaaaacccaaggacaccctcatgatctcccggacccctgaggtcacatgcgtggtggtggacgtgagccacgaagaccctgaggtcaagttcaactggtacgtggacggcgtggaggtgcataatgccaagacaaagccgcgggaggagcagtacaacagcacgtaccgtgtggtcagcgtcctcaccgtcctgcaccaggactggctgaatggcaaggagtacaagtgcaaggtctccaacaaagccctcccagcccccatcgagaaaaccatctccaaagccaaagggcagccccgagaaccacaggtgtacaccctgcccccatcccgggatgagctgaccaagaaccaggtcagcctgacctgcctggtcaaaggcttctatcccagcgacatcgccgtggagtgggagagcaatgggcagccggagaacaactacaagaccacgcctcccgtgctggactccgacggctccttcttcctctacagcaagctcaccgtggacaagagcaggtggcagcaggggaacgtcttctcatgctccgtgatgcatgaggctctgcacaaccactacacgcagaagagcctctccctgtctccgggtaaa

SEQ ID NO: 69 - DNA, 36 bp, synthetic construct
  source 1..36: mol_type = other DNA
gcctccggactctagagggccaccatgctgctgtcg

SEQ ID NO: 70 - DNA, 41 bp, synthetic construct
  source 1..41: mol_type = other DNA
tccggcggaggtggaagcgaagtccagctggtggaaagtgg

SEQ ID NO: 71 - DNA, 41 bp, synthetic construct
  source 1..41: mol_type = other DNA
ccactttccaccagctggacttcgcttccacctccgccgga

SEQ ID NO: 72 - DNA, 42 bp, synthetic construct; identical to SEQ ID NO: 54
  source 1..42: mol_type = other DNA

SEQ ID NO: 73 - DNA, 36 bp, synthetic construct; identical to SEQ ID NO: 69
  source 1..36: mol_type = other DNA

SEQ ID NO: 74 - DNA, 44 bp, synthetic construct
  source 1..44: mol_type = other DNA
tccggcggaggtggaagcgatatacagatgacgcagagccctag

SEQ ID NO: 75 - DNA, 44 bp, synthetic construct
  source 1..44: mol_type = other DNA
ctagggctctgcgtcatctgtatatcgcttccacctccgccgga

SEQ ID NO: 76 - DNA, 43 bp, synthetic construct; identical to SEQ ID NO: 52
  source 1..43: mol_type = other DNA

SEQ ID NO: 77 - DNA, 39 bp, synthetic construct
  source 1..39: mol_type = other DNA
gcctccggactctagagggtacgggccagatatacgcgt

SEQ ID NO: 78 - DNA, 45 bp, synthetic construct
  source 1..45: mol_type = other DNA
cattactaaccggtagggtcatttagctctgtgtggtaagcaggt

SEQ ID NO: 79 - DNA, 21 bp, synthetic construct
  source 1..21: mol_type = other DNA
cgcaaatgggcggtaggcgtg

SEQ ID NO: 80 - DNA, 60 bp, synthetic construct
  source 1..60: mol_type = other DNA
atgctgctgtcgccgtcgctgctgctgctgctgctgctgggggcgccgcggggctgcgcc

SEQ ID NO: 81 - DNA, 60 bp, synthetic construct
  source 1..60: mol_type = other DNA
atgagtgtgcccactcaggtcctggggttgctgctgctgtggcttacagatgccagatgt

SEQ ID NO: 82 - DNA, 57 bp, synthetic construct
  source 1..57: mol_type = other DNA
atggaatggagctgggtctttctcttcttcctgtcagtaactacaggtgtccactcc

SEQ ID NO: 83 - protein, 11 aa, synthetic construct
RASQDVGTAVA

SEQ ID NO: 84 - protein, 7 aa, synthetic construct
SASGLYS

SEQ ID NO: 85 - protein, 9 aa, synthetic construct
QQHGTTPPT

SEQ ID NO: 86 - protein, 10 aa, synthetic construct
GFNIKDTYIH

SEQ ID NO: 87 - protein, 15 aa, synthetic construct
RIYPTNGGTRYADSV

SEQ ID NO: 88 - protein, 11 aa, synthetic construct
WGGDGFGAMDY

SEQ ID NO: 89 - protein, 10 aa, synthetic construct
GFNIKDTGIH

SEQ ID NO: 90 - protein, 15 aa, synthetic construct
GIYPTNGGTGYADSV

SEQ ID NO: 91 - protein, 11 aa, synthetic construct
GGGDGFGAMDY

SEQ ID NO: 92 - protein, 355 aa, synthetic construct
EGVAAALTPERLLEWQDKGIFVIQSESLKKCIQAGKSVLTLENCKQANKHMLWKWVSNHGLFNIGGSGCLGLNFSAPEQPLSLYECDSTLVSLRWRCNRKMITGPLQYSVQVAHDNTVVASRKYIHKWISYGSGGGDICEYLHKDLHTIKGNTHGMPCMFPFQYNHQWHHECTREGREDDLLWCATTSRYERDEKWGFCPDPTSAEVGCDTIWEKDLNSHICYQFNLLSSLSWSEAHSSCQMQGGTLLSITDETEENFIREHMSSKTVEVWMGLNQLDEHAGWQWSDGTPLNYLNWSPEVNFEPFVEDHCGTFSSFMPSAWRSRDCESTLPYICKKYLNHIDHEIVEGGHHHHHH

SEQ ID NO: 93 - DNA, 1065 bp, synthetic construct
  source 1..1065: mol_type = other DNA
gagggtgtggcggcggcgcttacccccgagcggctcctggagtggcaggataaaggaatatttgttatccaaagtgagagtctcaagaaatgcattcaagcaggtaaatcggttctgaccctggagaactgcaagcaagcaaacaagcacatgctgtggaaatgggtttcaaaccatggcctctttaacataggaggcagtggttgcctgggcctgaatttctccgccccagagcagccattaagcttatatgaatgtgactccaccctcgtttccttacggtggcgctgtaacaggaagatgatcacaggcccgctgcagtactctgtccaggtggcgcatgacaacacagtggtggcctcacggaagtatattcataagtggatttcttatgggtcaggtggtggagacatttgtgaatatctacacaaagatttgcatacaatcaaagggaacacccacgggatgccgtgtatgtttcccttccagtataaccatcagtggcatcatgaatgtacccgtgaaggtcgggaagatgacttactgtggtgtgccacgacaagccgttatgaaagagatgaaaagtggggattttgccctgatcccacctctgcagaagtaggttgtgatactatttgggagaaggacctcaattcacacatttgctaccagttcaacctgctttcatctctctcttggagtgaggcacattcttcatgccagatgcaaggaggtacgctgttaagtattacagatgaaactgaagaaaatttcataagggagcacatgagcagtaaaacagtggaggtgtggatgggcctcaatcagctggatgaacacgctggctggcagtggtctgatggaacgccgctcaactatctgaattggagcccagaggtaaattttgagccatttgttgaagatcactgtggaacatttagttcatttatgccaagtgcctggaggagtcgggattgtgagtccaccttgccatatatatgtaaaaaatatctaaaccacattgatcatgaaatagttgaaggaggtcatcaccatcaccatcac

SEQ ID NO: 94 - skipped

SEQ ID NO: 95 - protein, 107 aa, synthetic construct
DIQMTQSPSSLSASVGDRVTITCRASQDVGTAVAWYQQKPGKAPKLLIYSASGLYSGVPSRFSGSRSGTDFTLTISSLQPEDFATYYCQQHGTTPPTFGQGTKVEIK

SEQ ID NO: 96 - protein, 118 aa, synthetic construct
EVQLVESGGGLVQPGGSLRLSCAASGFNIKDTYIHWVRQAPGKGLEWVARIYPTNGGTRYADSVKGRFTISADTSKNTAYLQMNSLRAEDTAVYYCSRWGGDGFGAMDYWGQGTLVTV

SEQ ID NO: 97 - protein, 118 aa, synthetic construct
EVQLVESGGGLVQPGGSLRLSCAASGFNIKDTGIHWVRQAPGKGLEWVAGIYPTNGGTGYADSVKGRFTISADTSKNTAYLQMNSLRAEDTAVYYCSRGGGDGFGAMDYWGQGTLVTV